European Patent Application EP 4 438 731 A1, published October 2, 2024. Title: FUSION PROTEIN COMPRISING SIRPα MUTANT. Applicant: 杭州尚健生物技术有限公司. The sequence listing filed with the application follows.

SEQUENCE LISTING (35 sequences)

SEQ ID NO: 1 - protein, 117 aa, synthetic construct
  REGION 1..117: note = M1N
ELQVIQPDKSVLVAAGETATLRCTATSLLPIGPIQWFRGAGPGRILIYNQKKGHFPRVTTLSDSTRRGNMDFSIRIGAITPADAGTYYCVKFRKGSPDDLEFKSGAGTELSVRAKPS

SEQ ID NO: 2 - protein, 117 aa, synthetic construct
  REGION 1..117: note = M5N
ELQVIQPDKSVLVAAGETATLRCTATSLVPVGPIQWFRGAGPGRNLIYNSRHGHFPRVTTVSDLTKRNNMDFSIRIGAITPADAGTYYCVKFRKGSPDDVEFKSGAGTELSVRAKPS

SEQ ID NO: 3 - protein, 117 aa, synthetic construct
  REGION 1..117: note = M12N
ELQVIQPDKSVLVAAGETATLRCTATSLFPIGPIQWFRGAGPGRELIYNQRKGHFPRVTTVSDLTKRNNMDFSIRIGAITPADAGTYYCVKFRKGSPDDIEFKSGAGTELSVRAKPS

SEQ ID NO: 4 - protein, 117 aa, synthetic construct
  REGION 1..117: note = M35N
ELQVIQPDKSVLVAAGETATLRCTATSLLPVGPIQWFRGAGPGRQLIYNQKDGHFPRVTTVSDLTKRNNMDFSINIGAITPADAGTYYCVKFRKGSPDDIEFKSGAGTELSVRAKPS

SEQ ID NO: 5 - protein, 117 aa, synthetic construct
  REGION 1..117: note = M37N
ELQVIQPDKSVLVAAGETATLRCTATSLLPIGPIQWFRGAGPGRKLIYNQRDGHFPRVTTVSDLTKRGNMDFSIRIGAITPADAGTYYCVKFRKGSPDDVEFKSGAGTELSVRAKPS

SEQ ID NO: 6 - protein, 117 aa, synthetic construct
  REGION 1..117: note = M41N
ELQVIQPDKSVLVAAGETATLRCTATSLVPVGPIQWFRGAGPGRHLIYNRRHGHFPRVTTVSDLTKRNNMDFSISIGAITPADAGTYYCVKFRKGSPDDVEFKSGAGTELSVRAKPS

SEQ ID NO: 7 - protein, 117 aa, synthetic construct
  REGION 1..117: note = M57N
ELQVIQPDKSVLVAAGETATLRCTATSLLPVGPIQWFRGAGPGRILIYNGKRGHFPRVTTLSDTTKRGNMDFSISIRAITPADAGTYYCVKFRKGSPDDREFKSGAGTELSVRAKPS

SEQ ID NO: 8 - protein, 117 aa, synthetic construct
  REGION 1..117: note = M67N
ELQVIQPDKSVLVAAGETATLRCTATSLLPVGPIQWFRGAGPGRMLIYNGRDGHFPRVTTVSDLTKRNNMDFSIRIGAITPADAGTYYCVKFRKGSPDDLEFKSGAGTELSVRAKPS

SEQ ID NO: 9 - protein, 117 aa, synthetic construct
  REGION 1..117: note = M81N
ELQVIQPDKSVLVAAGETATLRCTATSLLPVGPIQWFRGAGPGRELIYNQKEGHFPRVTTVSDLTKRNNMDFSIRIGAITPADAGTYYCVKFRKGSPDDVEFKSGAGTELSVRAKPS

SEQ ID NO: 10 - protein, 117 aa, synthetic construct
  REGION 1..117: note = M82N
ELQVIQPDKSVLVAAGETATLRCTATSLFPVGPIQWFRGAGPGRELIYNQKEGHFPRVTTVSHSTKRNNMDFSIRIHAITPADAGTYYCVKFRKGSPDDSEFKSGAGTELSVRAKPS

SEQ ID NO: 11 - protein, 117 aa, synthetic construct
  REGION 1..117: note = M84N
ELQVIQPDKSVLVAAGETATLRCTATSLFPVGPIQWFRGAGPGRELIYNQKEGHFPRVTTVSHSTRRNNMDFSIRIHAITPADAGTYYCVKFRKGSPDDSEFKSGAGTELSVRAKPS

SEQ ID NO: 12 - protein, 117 aa, synthetic construct
  REGION 1..117: note = M91N
ELQVIQPDKSVLVAAGETATLRCTATSLLPVGPIQWFRGAGPGRQLIYNQKDGHFPRVTTASDLTKRNNMDFSINIGAITPADAGTYYCVKFRKGSPDDIEFKSGAGTELSVRAKPS

SEQ ID NO: 13 - protein, 117 aa, synthetic construct
  REGION 1..117: note = M99N
ELQVIQPDKSVLVAAGETATLRCTATSLIPVGPIQWFRGAGPGRKLIYNQKEGHFPRVTTVSDSTKRKNMDFSIRIHAITPADAGTYYCVKFRKGSPDDLEFKSGAGTELSVRAKPS

SEQ ID NO: 14 - protein, 117 aa, synthetic construct
  REGION 1..117: note = M102N
ELQVIQPDKSVLVAAGETATLRCTATSLLPIGPIQWFRGAGPGRELIYNGKGGHFPRVTTVSRSTKRDNMDFSIRIGAITPADAGTYYCVKFRKGSPDDIEFKSGAGTELSVRAKPS

SEQ ID NO: 15 - protein, 117 aa, synthetic construct
  REGION 1..117: note = M111N
ELQVIQPDKSVLVAAGETATLRCTATSLLPVGPIQWFRGAGPGRRLIYNNRGGHFPRVTTLSETTRRDNMDFSIRIGAITPADAGTYYCVKFRKGSPDDLEFKSGAGTELSVRAKPS

SEQ ID NO: 16 - protein, 117 aa, synthetic construct
  REGION 1..117: note = M122N
ELQVIQPDKSVLVAAGETATLRCTATSLVPVGPIQWFRGAGPGRNLIYNSRHGHFPRVTTASDLTKRNNMDFSIRIGAITPADAGTYYCVKFRKGSPDDVEFKSGAGTELSVRAKPS

SEQ ID NO: 17 - protein, 117 aa, synthetic construct
  REGION 1..117: note = M126N
ELQVIQPDKSVLVAAGETATLRCTATSLVPIGPIQWFRGAGPGRVLIYNQRDGHFPRVTTVSETTRRENMDFSIRIGAITPADAGTYYCVKFRKGSPDDVEFKSGAGTELSVRAKPS

SEQ ID NO: 18 - protein, 117 aa, synthetic construct
  REGION 1..117: note = M130N
ELQVIQPDKSVLVAAGETATLRCTATSLLPIGPIQWFRGAGPGRVLIYNQREGHFPRVTTVSESTRRDNMDFSIRIRAITPADAGTYYCVKFRKGSPDDVEFKSGAGTELSVRAKPS

SEQ ID NO: 19 - protein, 117 aa, synthetic construct
  REGION 1..117: note = M135N
ELQVIQPDKSVLVAAGETATLRCTATSLVPVGPIQWFRGAGPGRLLIYNGKGGHFPRVTTLSETTRRGNMDFSIRIGAITPADAGTYYCVKFRKGSPDDVEFKSGAGTELSVRAKPS

SEQ ID NO: 20 - protein, 117 aa, synthetic construct
  REGION 1..117: note = M145N
ELQVIQPDKSVLVAAGETATLRCTATSLLPIGPIQWFRGAGPGRNLIYNGKGGHFPRVTTVSDLTKRNNMDFSIRIGAITPADAGTYYCVKFRKGSPDDVEFKSGAGTELSVRAKPS

SEQ ID NO: 21 - protein, 117 aa, synthetic construct
  REGION 1..117: note = M169N
ELQVIQPDKSVVVAAGETATLRCTATSLFPVGPIQWFRGAGPGRILIYNRRQGHFPRVTTVSDLTKRNNMDFSIRIGAITPADAGTYYCVKFRKGSPDDIEFKSGAGTELSVRAKPS

SEQ ID NO: 22 - protein, 504 aa, synthetic construct
  REGION 1..504: note = human SIRPa variant 1
MEPAGPAPGRLGPLLCLLLAASCAWSGVAGEEELQVIQPDKSVLVAAGETATLRCTATSLIPVGPIQWFRGAGPGRELIYNQKEGHFPRVTTVSDLTKRNNMDFSIRIGNITPADAGTYYCVKFRKGSPDDVEFKSGAGTELSVRAKPSAPVVSGPAARATPQHTVSFTCESHGFSPRDITLKWFKNGNELSDFQTNVDPVGESVSYSIHSTAKVVLTREDVHSQVICEVAHVTLQGDPLRGTANLSETIRVPPTLEVTQQPVRAENQVNVTCQVRKFYPQRLQLTWLENGNVSRTETASTVTENKDGTYNWMSWLLVNVSAHRDDVKLTCQVEHDGQPAVSKSHDLKVSAHPKEQGSNTAAENTGSNERNIYIVVGVVCTLLVALLMAALYLVRIRQKKAQGSTSSTRLHEPEKNAREITQDTNDITYADLNLPKGKKPAPQAAEPNNHTEYASIQTSPQPASEDTLTYADLDMVHLNRTPKQPAPKPEPSFSEYASVQVPRK

SEQ ID NO: 23 - protein, 117 aa, synthetic construct
  REGION 1..117: note = human wildtype SIRPa truncated domain (positions 33-149)
ELQVIQPDKSVLVAAGETATLRCTATSLIPVGPIQWFRGAGPGRELIYNQKEGHFPRVTTVSDLTKRNNMDFSIRIGNITPADAGTYYCVKFRKGSPDDVEFKSGAGTELSVRAKPS

SEQ ID NO: 24 - protein, 120 aa, synthetic construct
  REGION 1..120: note = CLDN18.2 VHH
QVQLVESGGGLVQPGGSLRLSCAASGSIFNIPVMGWYRQAPGKQRELVAGISTGGTTNYGDSVKGRFTISRDNAKNTVYLQMNSLKPEDTAVYYCNVLVVSGIGSTLEVWGQGTLVTVSS

SEQ ID NO: 25 - protein, 14 aa, synthetic construct
  REGION 1..14: note = HCDR3 (IMGT)
NVLVVSGIGSTLEV

SEQ ID NO: 26 - protein, 7 aa, synthetic construct
  REGION 1..7: note = HCDR2 (IMGT)
ISTGGTT

SEQ ID NO: 27 - protein, 8 aa, synthetic construct
  REGION 1..8: note = HCDR1 (IMGT)
GSIFNIPV

SEQ ID NO: 28 - protein, 232 aa, synthetic construct
  REGION 1..232: note = IgG1-Fc
EPKSCDKTHTCPPCPAPELLGGPSVFLFPPKPKDTLMISRTPEVTCVVVDVSHEDPEVKFNWYVDGVEVHNAKTKPREEQYNSTYRVVSVLTVLHQDWLNGKEYKCKVSNKALPAPIEKTISKAKGQPREPQVYTLPPSRDELTKNQVSLTCLVKGFYPSDIAVEWESNGQPENNYKTTPPVLDSDGSFFLYSKLTVDKSRWQQGNVFSCSVMHEALHNHYTQKSLSLSPGK

SEQ ID NO: 29 - protein, 10 aa, synthetic construct
  REGION 1..10: note = linker
GGGGSGGGGS

SEQ ID NO: 30 - protein, 479 aa, synthetic construct
  REGION 1..479: note = CS001
QVQLVESGGGLVQPGGSLRLSCAASGSIFNIPVMGWYRQAPGKQRELVAGISTGGTTNYGDSVKGRFTISRDNAKNTVYLQMNSLKPEDTAVYYCNVLVVSGIGSTLEVWGQGTLVTVSSEPKSCDKTHTCPPCPAPELLGGPSVFLFPPKPKDTLMISRTPEVTCVVVDVSHEDPEVKFNWYVDGVEVHNAKTKPREEQYNSTYRVVSVLTVLHQDWLNGKEYKCKVSNKALPAPIEKTISKAKGQPREPQVYTLPPSRDELTKNQVSLTCLVKGFYPSDIAVEWESNGQPENNYKTTPPVLDSDGSFFLYSKLTVDKSRWQQGNVFSCSVMHEALHNHYTQKSLSLSPGKGGGGSGGGGSELQVIQPDKSVLVAAGETATLRCTATSLLPVGPIQWFRGAGPGRQLIYNQKDGHFPRVTTASDLTKRNNMDFSINIGAITPADAGTYYCVKFRKGSPDDIEFKSGAGTELSVRAKPS

SEQ ID NO: 31 - protein, 479 aa, synthetic construct
  REGION 1..479: note = CS002
QVQLVESGGGLVQPGGSLRLSCAASGSIFNIPVMGWYRQAPGKQRELVAGISTGGTTNYGDSVKGRFTISRDNAKNTVYLQMNSLKPEDTAVYYCNVLVVSGIGSTLEVWGQGTLVTVSSEPKSCDKTHTCPPCPAPELLGGPSVFLFPPKPKDTLMISRTPEVTCVVVDVSHEDPEVKFNWYVDGVEVHNAKTKPREEQYNSTYRVVSVLTVLHQDWLNGKEYKCKVSNKALPAPIEKTISKAKGQPREPQVYTLPPSRDELTKNQVSLTCLVKGFYPSDIAVEWESNGQPENNYKTTPPVLDSDGSFFLYSKLTVDKSRWQQGNVFSCSVMHEALHNHYTQKSLSLSPGKGGGGSGGGGSELQVIQPDKSVLVAAGETATLRCTATSLIPVGPIQWFRGAGPGRELIYNQKEGHFPRVTTVSDLTKRNNMDFSIRIGAITPADAGTYYCVKFRKGSPDDVEFKSGAGTELSVRAKPS

SEQ ID NO: 32 - protein, 479 aa, synthetic construct
  REGION 1..479: note = CS003
QVQLVESGGGLVQPGGSLRLSCAASGSIFNIPVMGWYRQAPGKQRELVAGISTGGTTNYGDSVKGRFTISRDNAKNTVYLQMNSLKPEDTAVYYCNVLVVSGIGSTLEVWGQGTLVTVSSEPKSCDKTHTCPPCPAPELLGGPSVFLFPPKPKDTLMISRTPEVTCVVVDVSHEDPEVKFNWYVDGVEVHNAKTKPREEQYNSTYRVVSVLTVLHQDWLNGKEYKCKVSNKALPAPIEKTISKAKGQPREPQVYTLPPSRDELTKNQVSLTCLVKGFYPSDIAVEWESNGQPENNYKTTPPVLDSDGSFFLYSKLTVDKSRWQQGNVFSCSVMHEALHNHYTQKSLSLSPGKGGGGSGGGGSELQVIQPDKSVLVAAGETATLRCTATSLVPVGPIQWFRGAGPGRNLIYNSRHGHFPRVTTVSDLTKRNNMDFSIRIGAITPADAGTYYCVKFRKGSPDDVEFKSGAGTELSVRAKPS

SEQ ID NO: 33 - protein, 479 aa, synthetic construct
  REGION 1..479: note = CS004
QVQLVESGGGLVQPGGSLRLSCAASGSIFNIPVMGWYRQAPGKQRELVAGISTGGTTNYGDSVKGRFTISRDNAKNTVYLQMNSLKPEDTAVYYCNVLVVSGIGSTLEVWGQGTLVTVSSEPKSCDKTHTCPPCPAPELLGGPSVFLFPPKPKDTLMISRTPEVTCVVVDVSHEDPEVKFNWYVDGVEVHNAKTKPREEQYNSTYRVVSVLTVLHQDWLNGKEYKCKVSNKALPAPIEKTISKAKGQPREPQVYTLPPSRDELTKNQVSLTCLVKGFYPSDIAVEWESNGQPENNYKTTPPVLDSDGSFFLYSKLTVDKSRWQQGNVFSCSVMHEALHNHYTQKSLSLSPGKGGGGSGGGGSELQVIQPDKSVVVAAGETATLRCTATSLFPVGPIQWFRGAGPGRILIYNRRQGHFPRVTTVSDLTKRNNMDFSIRIGAITPADAGTYYCVKFRKGSPDDIEFKSGAGTELSVRAKPS

SEQ ID NO: 34 - protein, 479 aa, synthetic construct
  REGION 1..479: note = CS005
QVQLVESGGGLVQPGGSLRLSCAASGSIFNIPVMGWYRQAPGKQRELVAGISTGGTTNYGDSVKGRFTISRDNAKNTVYLQMNSLKPEDTAVYYCNVLVVSGIGSTLEVWGQGTLVTVSSEPKSCDKTHTCPPCPAPELLGGPSVFLFPPKPKDTLMISRTPEVTCVVVDVSHEDPEVKFNWYVDGVEVHNAKTKPREEQYNSTYRVVSVLTVLHQDWLNGKEYKCKVSNKALPAPIEKTISKAKGQPREPQVYTLPPSRDELTKNQVSLTCLVKGFYPSDIAVEWESNGQPENNYKTTPPVLDSDGSFFLYSKLTVDKSRWQQGNVFSCSVMHEALHNHYTQKSLSLSPGKGGGGSGGGGSELQVIQPDKSVLVAAGETATLRCTATSLFPVGPIQWFRGAGPGRELIYNQKEGHFPRVTTVSHSTKRNNMDFSIRIHAITPADAGTYYCVKFRKGSPDDSEFKSGAGTELSVRAKPS

SEQ ID NO: 35 - protein, 479 aa, synthetic construct
  REGION 1..479: note = CS006
QVQLVESGGGLVQPGGSLRLSCAASGSIFNIPVMGWYRQAPGKQRELVAGISTGGTTNYGDSVKGRFTISRDNAKNTVYLQMNSLKPEDTAVYYCNVLVVSGIGSTLEVWGQGTLVTVSSEPKSCDKTHTCPPCPAPELLGGPSVFLFPPKPKDTLMISRTPEVTCVVVDVSHEDPEVKFNWYVDGVEVHNAKTKPREEQYNSTYRVVSVLTVLHQDWLNGKEYKCKVSNKALPAPIEKTISKAKGQPREPQVYTLPPSRDELTKNQVSLTCLVKGFYPSDIAVEWESNGQPENNYKTTPPVLDSDGSFFLYSKLTVDKSRWQQGNVFSCSVMHEALHNHYTQKSLSLSPGKGGGGSGGGGSELQVIQPDKSVLVAAGETATLRCTATSLFPVGPIQWFRGAGPGRELIYNQKEGHFPRVTTVSHSTRRNNMDFSIRIHAITPADAGTYYCVKFRKGSPDDSEFKSGAGTELSVRAKPS